European Patent Application EP 4 194 473 A1, published June 14, 2023. Title: Construction of chimeric antigen receptor targeting CD20 antigen and activity identification of engineered T cells thereof. Applicant: CELLULAR BIOMEDICINE GROUP (HK) LTD. The sequence listing filed with the application follows.

SEQUENCE LISTING (40 sequences)

SEQ ID NO: 1 - protein, 672 aa, synthetic construct
  REGION 1..672: note = CAR
MALPVTALLLPLALLLHAARPEVQLVESGGGLVQPGRSLRLSCAASGFTFNDYAMHWVRQAPGKGLEWVSTISWNSGSIGYADSVKGRFTISRDNAKKSLYLQMNSLRAEDTALYYCAKDIQYGNYYYGMDVWGQGTTVTVSSGGGGSGGGGSGGGGSEIVLTQSPATLSLSPGERATLSCRASQSVSSYLAWYQQKPGQAPRLLIYDASNRATGIPARFSGSGSGTDFTLTISSLEPEDFAVYYCQQRSNWPITFGQGTRLEIKESKYGPPCPPCPAPEFLGGPSVFLFPPKPKDTLMISRTPEVTCVVVDVSQEDPEVQFNWYVDGVEVHNAKTKPREEQFNSTYRVVSVLTVLHQDWLNGKEYKCKVSNKGLPSSIEKTISKAKGQPREPQVYTLPPSQEEMTKNQVSLTCLVKGFYPSDIAVEWESNGQPENNYKTTPPVLDSDGSFFLYSRLTVDKSRWQEGNVFSCSVMHEALHNHYTQKSLSLSLGKIYIWAPLAGTCGVLLLSLVITLYCKRGRKKLLYIFKQPFMRPVQTTQEEDGCSCRFPEEEEGGCELRVKFSRSADAPAYKQGQNQLYNELNLGRREEYDVLDKRRGRDPEMGGKPRRKNPQEGLYNELQKDKMAEAYSEIGMKGERRRGKGHDGLYQGLSTATKDTYDALHMQALPPR

SEQ ID NO: 2 - DNA, 2019 bp, synthetic construct
  misc_feature 1..2019: note = CAR
  source 1..2019: mol_type = other DNA
atggccttaccagtgaccgccttgctcctgccgctggccttgctgctccacgccgccaggccggaagtgcagctggtggagtctgggggaggcttggtacagcctggcaggtccctgagactctcctgtgcagcctctggattcacctttaatgattatgccatgcactgggtccggcaagctccagggaagggcctggagtgggtctcaactattagttggaatagtggttccataggctatgcggactctgtgaagggccgattcaccatctccagagacaacgccaagaagtccctgtatctgcaaatgaacagtctgagagctgaggacacggccttgtattactgtgcaaaagatatacagtacggcaactactactacggtatggacgtctggggccaagggaccacggtcaccgtctcctcaggtggcggtggctcgggcggtggtgggtcgggtggcggcggatctgaaattgtgttgacacagtctccagccaccctgtctttgtctccaggggaaagagccaccctctcctgcagggccagtcagagtgttagcagctacttagcctggtaccaacagaaacctggccaggctcccaggctcctcatctatgatgcatccaacagggccactggcatcccagccaggttcagtggcagtgggtctgggacagacttcactctcaccatcagcagcctagagcctgaagattttgcagtttattactgtcagcagcgtagcaactggccgatcaccttcggccaagggacacgactggagattaaagagagcaagtacggaccgccctgccccccttgccctgcccccgagttcctgggcggacccagcgtgttcctgttcccccccaagcccaaggacaccctgatgatcagccggacccccgaggtgacctgcgtggtggtggacgtgagccaggaagatcccgaggtccagttcaattggtacgtggacggcgtggaagtgcacaacgccaagaccaagcccagagaggaacagttcaacagcacctaccgggtggtgtctgtgctgaccgtgctgcaccaggactggctgaacggcaaagaatacaagtgcaaggtgtccaacaagggcctgcccagcagcatcgaaaagaccatcagcaaggccaagggccagcctcgcgagccccaggtgtacaccctgcctccctcccaggaagagatgaccaagaaccaggtgtccctgacctgcctggtgaagggcttctaccccagcgacatcgccgtggagtgggagagcaacggccagcctgagaacaactacaagaccacccctcccgtgctggacagcgacggcagcttcttcctgtacagccggctgaccgtggacaagagccggtggcaggaaggcaacgtctttagctgcagcgtgatgcacgaggccctgcacaaccactacacccagaagagcctgagcctgtccctgggcaagatctacatctgggcgcccttggccgggacttgtggggtccttctcctgtcactggttatcaccctttactgcaaacggggcagaaagaaactcctgtatatattcaaacaaccatttatgagaccagtacaaactactcaagaggaagatggctgtagctgccgatttccagaagaagaagaaggaggatgtgaactgagagtgaagttcagcaggagcgcagacgcccccgcgtacaagcagggccagaaccagctctataacgagctcaatctaggacgaagagaggagtacgatgttttggacaagagacgtggccgggaccctgagatggggggaaagccgagaaggaagaaccctcaggaaggcctgtacaatgaactgcagaaagataagatggcggaggcctacagtgagattgggatgaaaggcgagcgccggaggggcaaggggcacgatggcctttaccagggtctcagtacagccaccaaggacacctacgacgcccttcacatgcaggccctgccccctcgctag

SEQ ID NO: 3 - protein, 670 aa, synthetic construct
  REGION 1..670: note = CAR
MALPVTALLLPLALLLHAARPQVQLQQPGAELVKPGASVKMSCKASGYTFTSYNMHWVKQTPGRGLEWIGAIYPGNGDTSYNQKFKGKATLTADKSSSTAYMQLSSLTSEDSAVYYCARSTYYGGDWYFNVWGAGTTVTVSAGGGGSGGGGSGGGGSQIVLSQSPAILSASPGEKVTMTCRASSSVSYIHWFQQKPGSSPKPWIYATSNLASGVPVRFSGSGSGTSYSLTISRVEAEDAATYYCQQWTSNPPTFGGGTKLEIKESKYGPPCPPCPAPEFLGGPSVFLFPPKPKDTLMISRTPEVTCVVVDVSQEDPEVQFNWYVDGVEVHNAKTKPREEQFNSTYRVVSVLTVLHQDWLNGKEYKCKVSNKGLPSSIEKTISKAKGQPREPQVYTLPPSQEEMTKNQVSLTCLVKGFYPSDIAVEWESNGQPENNYKTTPPVLDSDGSFFLYSRLTVDKSRWQEGNVFSCSVMHEALHNHYTQKSLSLSLGKIYIWAPLAGTCGVLLLSLVITLYCKRGRKKLLYIFKQPFMRPVQTTQEEDGCSCRFPEEEEGGCELRVKFSRSADAPAYKQGQNQLYNELNLGRREEYDVLDKRRGRDPEMGGKPRRKNPQEGLYNELQKDKMAEAYSEIGMKGERRRGKGHDGLYQGLSTATKDTYDALHMQALPPR

SEQ ID NO: 4 - DNA, 2013 bp, synthetic construct
  misc_feature 1..2013: note = CAR
  source 1..2013: mol_type = other DNA
atggccttaccagtgaccgccttgctcctgccgctggccttgctgctccacgccgccaggccgcaggtgcagttgcaacagcctggagctgagttggtgaagcctggtgcttctgtgaagatgtcttgtaaggcttctggatacacattcacttcttacaacatgcactgggtgaagcagactcctggtaggggtttggagtggatcggagctatctacccaggaaacggagacacatcttacaaccagaagttcaagggtaaggctacattgactgctgacaagtcttcatctactgcttacatgcaattgtcttctttgacatctgaggactctgcagtttactactgcgctaggtctacatactacggaggtgactggtacttcaacgtgtggggagcaggtaccacggtcactgtctctgcaggtggaggtggatctggaggaggaggatctggtggaggaggttctcaaattgttctctcccagtctccagcaatcctgtcagcttctcctggagagaaggtgactatgacttgcagggcttcttcatctgtttcttacatccactggttccagcagaagcctggttcttcacctaagccttggatctacgctacatctaacttggcatctggagtgcctgtgaggttctctggttctggttcaggtacttcttactctttgacaatctctagggtggaggctgaggacgctgctacttactactgccagcagtggacatctaaccctccaacattcggaggtggtactaagttggagatcaaggagagcaagtacggaccgccctgccccccttgccctgcccccgagttcctgggcggacccagcgtgttcctgttcccccccaagcccaaggacaccctgatgatcagccggacccccgaggtgacctgcgtggtggtggacgtgagccaggaagatcccgaggtccagttcaattggtacgtggacggcgtggaagtgcacaacgccaagaccaagcccagagaggaacagttcaacagcacctaccgggtggtgtctgtgctgaccgtgctgcaccaggactggctgaacggcaaagaatacaagtgcaaggtgtccaacaagggcctgcccagcagcatcgaaaagaccatcagcaaggccaagggccagcctcgcgagccccaggtgtacaccctgcctccctcccaggaagagatgaccaagaaccaggtgtccctgacctgcctggtgaagggcttctaccccagcgacatcgccgtggagtgggagagcaacggccagcctgagaacaactacaagaccacccctcccgtgctggacagcgacggcagcttcttcctgtacagccggctgaccgtggacaagagccggtggcaggaaggcaacgtctttagctgcagcgtgatgcacgaggccctgcacaaccactacacccagaagagcctgagcctgtccctgggcaagatctacatctgggcgcccttggccgggacttgtggggtccttctcctgtcactggttatcaccctttactgcaaacggggcagaaagaaactcctgtatatattcaaacaaccatttatgagaccagtacaaactactcaagaggaagatggctgtagctgccgatttccagaagaagaagaaggaggatgtgaactgagagtgaagttcagcaggagcgcagacgcccccgcgtacaagcagggccagaaccagctctataacgagctcaatctaggacgaagagaggagtacgatgttttggacaagagacgtggccgggaccctgagatggggggaaagccgagaaggaagaaccctcaggaaggcctgtacaatgaactgcagaaagataagatggcggaggcctacagtgagattgggatgaaaggcgagcgccggaggggcaaggggcacgatggcctttaccagggtctcagtacagccaccaaggacacctacgacgcccttcacatgcaggccctgccccctcgctag

SEQ ID NO: 5 - protein, 672 aa, synthetic construct
  REGION 1..672: note = CAR
MALPVTALLLPLALLLHAARPEVQLVESGGGLVQPGRSLRLSCAASGFTFNDYAMHWVRQAPGKGLEWVSTISWNSGSIGYADSVKGRFTISRDNAKKSLYLQMNSLRAEDTALYYCAKDIQYGNYYYGMDVWGQGTTVTVSSGGGGSGGGGSGGGGSEIVLTQSPATLSLSPGERATLSCRASQSVSSYLAWYQQKPGQAPRLLIYDASNRATGIPARFSGSGSGTDFTLTISSLEPEDFAVYYCQQRSNWPITFGQGTRLEIKESKYGPPCPPCPAPEFEGGPSVFLFPPKPKDTLMISRTPEVTCVVVDVSQEDPEVQFNWYVDGVEVHNAKTKPREEQFQSTYRVVSVLTVLHQDWLNGKEYKCKVSNKGLPSSIEKTISKAKGQPREPQVYTLPPSQEEMTKNQVSLTCLVKGFYPSDIAVEWESNGQPENNYKTTPPVLDSDGSFFLYSRLTVDKSRWQEGNVFSCSVMHEALHNHYTQKSLSLSLGKIYIWAPLAGTCGVLLLSLVITLYCKRGRKKLLYIFKQPFMRPVQTTQEEDGCSCRFPEEEEGGCELRVKFSRSADAPAYKQGQNQLYNELNLGRREEYDVLDKRRGRDPEMGGKPRRKNPQEGLYNELQKDKMAEAYSEIGMKGERRRGKGHDGLYQGLSTATKDTYDALHMQALPPR

SEQ ID NO: 6 - DNA, 2019 bp, synthetic construct
  misc_feature 1..2019: note = CAR
  source 1..2019: mol_type = other DNA
atggccttaccagtgaccgccttgctcctgccgctggccttgctgctccacgccgccaggccggaagtgcagctggtggagtctgggggaggcttggtacagcctggcaggtccctgagactctcctgtgcagcctctggattcacctttaatgattatgccatgcactgggtccggcaagctccagggaagggcctggagtgggtctcaactattagttggaatagtggttccataggctatgcggactctgtgaagggccgattcaccatctccagagacaacgccaagaagtccctgtatctgcaaatgaacagtctgagagctgaggacacggccttgtattactgtgcaaaagatatacagtacggcaactactactacggtatggacgtctggggccaagggaccacggtcaccgtctcctcaggtggcggtggctcgggcggtggtgggtcgggtggcggcggatctgaaattgtgttgacacagtctccagccaccctgtctttgtctccaggggaaagagccaccctctcctgcagggccagtcagagtgttagcagctacttagcctggtaccaacagaaacctggccaggctcccaggctcctcatctatgatgcatccaacagggccactggcatcccagccaggttcagtggcagtgggtctgggacagacttcactctcaccatcagcagcctagagcctgaagattttgcagtttattactgtcagcagcgtagcaactggccgatcaccttcggccaagggacacgactggagattaaagagagcaagtacggaccgccctgccccccttgccctgcccccgagttcgagggcggacccagcgtgttcctgttcccccccaagcccaaggacaccctgatgatcagccggacccccgaggtgacctgcgtggtggtggacgtgagccaggaagatcccgaggtccagttcaattggtacgtggacggcgtggaagtgcacaacgccaagaccaagcccagagaggaacagttccaaagcacctaccgggtggtgtctgtgctgaccgtgctgcaccaggactggctgaacggcaaagaatacaagtgcaaggtgtccaacaagggcctgcccagcagcatcgaaaagaccatcagcaaggccaagggccagcctcgcgagccccaggtgtacaccctgcctccctcccaggaagagatgaccaagaaccaggtgtccctgacctgcctggtgaagggcttctaccccagcgacatcgccgtggagtgggagagcaacggccagcctgagaacaactacaagaccacccctcccgtgctggacagcgacggcagcttcttcctgtacagccggctgaccgtggacaagagccggtggcaggaaggcaacgtctttagctgcagcgtgatgcacgaggccctgcacaaccactacacccagaagagcctgagcctgtccctgggcaagatctacatctgggcgcccttggccgggacttgtggggtccttctcctgtcactggttatcaccctttactgcaaacggggcagaaagaaactcctgtatatattcaaacaaccatttatgagaccagtacaaactactcaagaggaagatggctgtagctgccgatttccagaagaagaagaaggaggatgtgaactgagagtgaagttcagcaggagcgcagacgcccccgcgtacaagcagggccagaaccagctctataacgagctcaatctaggacgaagagaggagtacgatgttttggacaagagacgtggccgggaccctgagatggggggaaagccgagaaggaagaaccctcaggaaggcctgtacaatgaactgcagaaagataagatggcggaggcctacagtgagattgggatgaaaggcgagcgccggaggggcaaggggcacgatggcctttaccagggtctcagtacagccaccaaggacacctacgacgcccttcacatgcaggccctgccccctcgctag

SEQ ID NO: 7 - protein, 122 aa, synthetic construct
  REGION 1..122: note = VH
EVQLVESGGGLVQPGRSLRLSCAASGFTFNDYAMHWVRQAPGKGLEWVSTISWNSGSIGYADSVKGRFTISRDNAKKSLYLQMNSLRAEDTALYYCAKDIQYGNYYYGMDVWGQGTTVTVSS

SEQ ID NO: 8 - DNA, 366 bp, synthetic construct
  misc_feature 1..366: note = VH
  source 1..366: mol_type = other DNA
gaagtgcagctggtggagtctgggggaggcttggtacagcctggcaggtccctgagactctcctgtgcagcctctggattcacctttaatgattatgccatgcactgggtccggcaagctccagggaagggcctggagtgggtctcaactattagttggaatagtggttccataggctatgcggactctgtgaagggccgattcaccatctccagagacaacgccaagaagtccctgtatctgcaaatgaacagtctgagagctgaggacacggccttgtattactgtgcaaaagatatacagtacggcaactactactacggtatggacgtctggggccaagggaccacggtcaccgtctcctca

SEQ ID NO: 9 - protein, 121 aa, synthetic construct [sequence omitted]

SEQ ID NO: 10 - DNA, 363 bp, synthetic construct
  misc_feature 1..363: note = VH
  source 1..363: mol_type = other DNA
caggtgcagttgcaacagcctggagctgagttggtgaagcctggtgcttctgtgaagatgtcttgtaaggcttctggatacacattcacttcttacaacatgcactgggtgaagcagactcctggtaggggtttggagtggatcggagctatctacccaggaaacggagacacatcttacaaccagaagttcaagggtaaggctacattgactgctgacaagtcttcatctactgcttacatgcaattgtcttctttgacatctgaggactctgcagtttactactgcgctaggtctacatactacggaggtgactggtacttcaacgtgtggggagcaggtaccacggtcactgtctctgca

SEQ ID NO: 11 - protein, 107 aa, synthetic construct
  REGION 1..107: note = VL
EIVLTQSPATLSLSPGERATLSCRASQSVSSYLAWYQQKPGQAPRLLIYDASNRATGIPARFSGSGSGTDFTLTISSLEPEDFAVYYCQQRSNWPITFGQGTRLEIK

SEQ ID NO: 12 - DNA, 321 bp, synthetic construct
  misc_feature 1..321: note = VL
  source 1..321: mol_type = other DNA
gaaattgtgttgacacagtctccagccaccctgtctttgtctccaggggaaagagccaccctctcctgcagggccagtcagagtgttagcagctacttagcctggtaccaacagaaacctggccaggctcccaggctcctcatctatgatgcatccaacagggccactggcatcccagccaggttcagtggcagtgggtctgggacagacttcactctcaccatcagcagcctagagcctgaagattttgcagtttattactgtcagcagcgtagcaactggccgatcaccttcggccaagggacacgactggagattaaa

SEQ ID NO: 13 - protein, 106 aa, synthetic construct [sequence omitted]

SEQ ID NO: 14 - DNA, 318 bp, synthetic construct
  misc_feature 1..318: note = VL
  source 1..318: mol_type = other DNA
caaattgttctctcccagtctccagcaatcctgtcagcttctcctggagagaaggtgactatgacttgcagggcttcttcatctgtttcttacatccactggttccagcagaagcctggttcttcacctaagccttggatctacgctacatctaacttggcatctggagtgcctgtgaggttctctggttctggttcaggtacttcttactctttgacaatctctagggtggaggctgaggacgctgctacttactactgccagcagtggacatctaaccctccaacattcggaggtggtactaagttggagatcaag

SEQ ID NO: 15 - protein, 15 aa, synthetic construct
  REGION 1..15: note = Linker Peptide
GGGGSGGGGSGGGGS

SEQ ID NO: 16 - DNA, 45 bp, synthetic construct
  misc_feature 1..45: note = Linker Peptide
  source 1..45: mol_type = other DNA
ggtggcggtggctcgggcggtggtgggtcgggtggcggcggatct

SEQ ID NO: 17 - protein, 229 aa, synthetic construct
  REGION 1..229: note = H
ESKYGPPCPPCPAPEFLGGPSVFLFPPKPKDTLMISRTPEVTCVVVDVSQEDPEVQFNWYVDGVEVHNAKTKPREEQFNSTYRVVSVLTVLHQDWLNGKEYKCKVSNKGLPSSIEKTISKAKGQPREPQVYTLPPSQEEMTKNQVSLTCLVKGFYPSDIAVEWESNGQPENNYKTTPPVLDSDGSFFLYSRLTVDKSRWQEGNVFSCSVMHEALHNHYTQKSLSLSLGK

SEQ ID NO: 18 - DNA, 687 bp, synthetic construct
  misc_feature 1..687: note = H
  source 1..687: mol_type = other DNA
gagagcaagtacggaccgccctgccccccttgccctgcccccgagttcctgggcggacccagcgtgttcctgttcccccccaagcccaaggacaccctgatgatcagccggacccccgaggtgacctgcgtggtggtggacgtgagccaggaagatcccgaggtccagttcaattggtacgtggacggcgtggaagtgcacaacgccaagaccaagcccagagaggaacagttcaacagcacctaccgggtggtgtctgtgctgaccgtgctgcaccaggactggctgaacggcaaagaatacaagtgcaaggtgtccaacaagggcctgcccagcagcatcgaaaagaccatcagcaaggccaagggccagcctcgcgagccccaggtgtacaccctgcctccctcccaggaagagatgaccaagaaccaggtgtccctgacctgcctggtgaagggcttctaccccagcgacatcgccgtggagtgggagagcaacggccagcctgagaacaactacaagaccacccctcccgtgctggacagcgacggcagcttcttcctgtacagccggctgaccgtggacaagagccggtggcaggaaggcaacgtctttagctgcagcgtgatgcacgaggccctgcacaaccactacacccagaagagcctgagcctgtccctgggcaag

SEQ ID NO: 19 - protein, 229 aa, synthetic construct
  REGION 1..229: note = H
ESKYGPPCPPCPAPEFEGGPSVFLFPPKPKDTLMISRTPEVTCVVVDVSQEDPEVQFNWYVDGVEVHNAKTKPREEQFQSTYRVVSVLTVLHQDWLNGKEYKCKVSNKGLPSSIEKTISKAKGQPREPQVYTLPPSQEEMTKNQVSLTCLVKGFYPSDIAVEWESNGQPENNYKTTPPVLDSDGSFFLYSRLTVDKSRWQEGNVFSCSVMHEALHNHYTQKSLSLSLGK

SEQ ID NO: 20 - DNA, 687 bp, synthetic construct
  misc_feature 1..687: note = H
  source 1..687: mol_type = other DNA
gagagcaagtacggaccgccctgccccccttgccctgcccccgagttcgagggcggacccagcgtgttcctgttcccccccaagcccaaggacaccctgatgatcagccggacccccgaggtgacctgcgtggtggtggacgtgagccaggaagatcccgaggtccagttcaattggtacgtggacggcgtggaagtgcacaacgccaagaccaagcccagagaggaacagttccaaagcacctaccgggtggtgtctgtgctgaccgtgctgcaccaggactggctgaacggcaaagaatacaagtgcaaggtgtccaacaagggcctgcccagcagcatcgaaaagaccatcagcaaggccaagggccagcctcgcgagccccaggtgtacaccctgcctccctcccaggaagagatgaccaagaaccaggtgtccctgacctgcctggtgaagggcttctaccccagcgacatcgccgtggagtgggagagcaacggccagcctgagaacaactacaagaccacccctcccgtgctggacagcgacggcagcttcttcctgtacagccggctgaccgtggacaagagccggtggcaggaaggcaacgtctttagctgcagcgtgatgcacgaggccctgcacaaccactacacccagaagagcctgagcctgtccctgggcaag

SEQ ID NO: 21 - protein, 24 aa, synthetic construct
  REGION 1..24: note = TM
IYIWAPLAGTCGVLLLSLVITLYC

SEQ ID NO: 22 - DNA, 72 bp, synthetic construct
  misc_feature 1..72: note = TM
  source 1..72: mol_type = other DNA
atctacatctgggcgcccttggccgggacttgtggggtccttctcctgtcactggttatcaccctttactgc

SEQ ID NO: 23 - protein, 42 aa, synthetic construct
  REGION 1..42: note = CS
KRGRKKLLYIFKQPFMRPVQTTQEEDGCSCRFPEEEEGGCEL

SEQ ID NO: 24 - DNA, 126 bp, synthetic construct
  misc_feature 1..126: note = CS
  source 1..126: mol_type = other DNA
aaacggggcagaaagaaactcctgtatatattcaaacaaccatttatgagaccagtacaaactactcaagaggaagatggctgtagctgccgatttccagaagaagaagaaggaggatgtgaactg

SEQ ID NO: 25 - protein, 113 aa, synthetic construct
  REGION 1..113: note = CD3zeta
RVKFSRSADAPAYQQGQNQLYNELNLGRREEYDVLDKRRGRDPEMGGKPQRRKNPQEGLYNELQKDKMAEAYSEIGMKGERRRGKGHDGLYQGLSTATKDTYDALHMQALPPR

SEQ ID NO: 26 - DNA, 336 bp, synthetic construct
  misc_feature 1..336: note = CD3zeta
  source 1..336: mol_type = other DNA
agagtgaagttcagcaggagcgcagacgcccccgcgtacaagcagggccagaaccagctctataacgagctcaatctaggacgaagagaggagtacgatgttttggacaagagacgtggccgggaccctgagatggggggaaagccgagaaggaagaaccctcaggaaggcctgtacaatgaactgcagaaagataagatggcggaggcctacagtgagattgggatgaaaggcgagcgccggaggggcaaggggcacgatggcctttaccagggtctcagtacagccaccaaggacacctacgacgcccttcacatgcaggccctgccccctcgc

SEQ ID NO: 27 - protein, 21 aa, synthetic construct
  REGION 1..21: note = L
MALPVTALLLPLALLLHAARP

SEQ ID NO: 28 - DNA, 63 bp, synthetic construct
  misc_feature 1..63: note = L
  source 1..63: mol_type = other DNA
atggccttaccagtgaccgccttgctcctgccgctggccttgctgctccacgccgccaggccg

SEQ ID NO: 29 - protein, 677 aa, synthetic construct
  REGION 1..677: note = CAR
MALPVTALLLPLALLLHAARPQVQLVQSGAEVKKPGSSVKVSCKASGYAFSYSWINWVRQAPGQGLEWMGRIFPGDGDTDYNGKFKGRVTITADKSTSTAYMELSSLRSEDTAVYYCARNVFDGYWLVYWGQGTLVTVSSGGGGSGGGGSGGGGSDIVMTQTPLSLPVTPGEPASISCRSSKSLLHSNGITYLYWYLQKPGQSPQLLIYQMSNLVSGVPDRFSGSGSGTDFTLKISRVEAEDVGVYYCAQNLELPYTFGGGTKVEIKRTVESKYGPPCPPCPAPEFLGGPSVFLFPPKPKDTLMISRTPEVTCVVVDVSQEDPEVQFNWYVDGVEVHNAKTKPREEQFNSTYRVVSVLTVLHQDWLNGKEYKCKVSNKGLPSSIEKTISKAKGQPREPQVYTLPPSQEEMTKNQVSLTCLVKGFYPSDIAVEWESNGQPENNYKTTPPVLDSDGSFFLYSRLTVDKSRWQEGNVFSCSVMHEALHNHYTQKSLSLSLGKIYIWAPLAGTCGVLLLSLVITLYCKRGRKKLLYIFKQPFMRPVQTTQEEDGCSCRFPEEEEGGCELRVKFSRSADAPAYKQGQNQLYNELNLGRREEYDVLDKRRGRDPEMGGKPRRKNPQEGLYNELQKDKMAEAYSEIGMKGERRRGKGHDGLYQGLSTATKDTYDALHMQALPPR

SEQ ID NO: 30 - DNA, 2034 bp, synthetic construct
  misc_feature 1..2034: note = CAR
  source 1..2034: mol_type = other DNA
atggccttaccagtgaccgccttgctcctgccgctggccttgctgctccacgccgccaggccgcaggtgcaattggtgcagtctggcgctgaagttaagaagcctgggagttcagtgaaggtctcctgcaaggcttccggatacgccttcagctattcttggatcaattgggtgcggcaggcgcctggacaagggctcgagtggatgggacggatctttcccggcgatggggatactgactacaatgggaaattcaagggcagagtcacaattaccgccgacaaatccactagcacagcctatatggagctgagcagcctgagatctgaggacacggccgtgtattactgtgcaagaaatgtctttgatggttactggcttgtttactggggccagggaaccctggtcaccgtctcctcaggtggcggtggctcgggcggtggtgggtcgggtggcggcggatctgatatcgtgatgacccagactccactctccctgcccgtcacccctggagagcccgccagcattagctgcaggtctagcaagagcctcttgcacagcaatggcatcacttatttgtattggtacctgcaaaagccagggcagtctccacagctcctgatttatcaaatgtccaaccttgtctctggcgtccctgaccggttctccggctccgggtcaggcactgatttcacactgaaaatcagcagggtggaggctgaggatgttggagtttattactgcgctcagaatctagaacttccttacaccttcggcggagggaccaaggtggagatcaaacgtacggtggagagcaagtacggaccgccctgccccccttgccctgcccccgagttcctgggcggacccagcgtgttcctgttcccccccaagcccaaggacaccctgatgatcagccggacccccgaggtgacctgcgtggtggtggacgtgagccaggaagatcccgaggtccagttcaattggtacgtggacggcgtggaagtgcacaacgccaagaccaagcccagagaggaacagttcaacagcacctaccgggtggtgtctgtgctgaccgtgctgcaccaggactggctgaacggcaaagaatacaagtgcaaggtgtccaacaagggcctgcccagcagcatcgaaaagaccatcagcaaggccaagggccagcctcgcgagccccaggtgtacaccctgcctccctcccaggaagagatgaccaagaaccaggtgtccctgacctgcctggtgaagggcttctaccccagcgacatcgccgtggagtgggagagcaacggccagcctgagaacaactacaagaccacccctcccgtgctggacagcgacggcagcttcttcctgtacagccggctgaccgtggacaagagccggtggcaggaaggcaacgtctttagctgcagcgtgatgcacgaggccctgcacaaccactacacccagaagagcctgagcctgtccctgggcaagatctacatctgggcgcccttggccgggacttgtggggtccttctcctgtcactggttatcaccctttactgcaaacggggcagaaagaaactcctgtatatattcaaacaaccatttatgagaccagtacaaactactcaagaggaagatggctgtagctgccgatttccagaagaagaagaaggaggatgtgaactgagagtgaagttcagcaggagcgcagacgcccccgcgtacaagcagggccagaaccagctctataacgagctcaatctaggacgaagagaggagtacgatgttttggacaagagacgtggccgggaccctgagatggggggaaagccgagaaggaagaaccctcaggaaggcctgtacaatgaactgcagaaagataagatggcggaggcctacagtgagattgggatgaaaggcgagcgccggaggggcaaggggcacgatggcctttaccagggtctcagtacagccaccaaggacacctacgacgcccttcacatgcaggccctgccccctcgctag

SEQ ID NO: 31 - protein, 716 aa, synthetic construct
  REGION 1..716: note = CAR
MALPVTALLLPLALLLHAARPEVQLVESGGGLVQPGRSLRLSCAASGFTFNDYAMHWVRQAPGKGLEWVSTISWNSGSIGYADSVKGRFTISRDNAKKSLYLQMNSLRAEDTALYYCAKDIQYGNYYYGMDVWGQGTTVTVSSGGGGSGGGGSGGGGSEIVLTQSPATLSLSPGERATLSCRASQSVSSYLAWYQQKPGQAPRLLIYDASNRATGIPARFSGSGSGTDFTLTISSLEPEDFAVYYCQQRSNWPITFGQGTRLEIKESKYGPPCPPCPAPEFEGGPSVFLFPPKPKDTLMISRTPEVTCVVVDVSQEDPEVQFNWYVDGVEVHNAKTKPREEQFQSTYRVVSVLTVLHQDWLNGKEYKCKVSNKGLPSSIEKTISKAKGQPREPQVYTLPPSQEEMTKNQVSLTCLVKGFYPSDIAVEWESNGQPENNYKTTPPVLDSDGSFFLYSRLTVDKSRWQEGNVFSCSVMHEALHNHYTQKSLSLSLGKFWVLVVVGGVLACYSLLVTVAFIIFWVRSKRSRLLHSDYMNMTPRRPGPTRKHYQPYAPPRDFAAYRSKRGRKKLLYIFKQPFMRPVQTTQEEDGCSCRFPEEEEGGCELRVKFSRSADAPAYKQGQNQLYNELNLGRREEYDVLDKRRGRDPEMGGKPRRKNPQEGLYNELQKDKMAEAYSEIGMKGERRRGKGHDGLYQGLSTATKDTYDALHMQALPPR

SEQ ID NO: 32 - DNA, 2151 bp, synthetic construct
  misc_feature 1..2151: note = CAR
  source 1..2151: mol_type = other DNA
atggccttaccagtgaccgccttgctcctgccgctggccttgctgctccacgccgccaggccggaagtgcagctggtggagtctgggggaggcttggtacagcctggcaggtccctgagactctcctgtgcagcctctggattcacctttaatgattatgccatgcactgggtccggcaagctccagggaagggcctggagtgggtctcaactattagttggaatagtggttccataggctatgcggactctgtgaagggccgattcaccatctccagagacaacgccaagaagtccctgtatctgcaaatgaacagtctgagagctgaggacacggccttgtattactgtgcaaaagatatacagtacggcaactactactacggtatggacgtctggggccaagggaccacggtcaccgtctcctcaggtggcggtggctcgggcggtggtgggtcgggtggcggcggatctgaaattgtgttgacacagtctccagccaccctgtctttgtctccaggggaaagagccaccctctcctgcagggccagtcagagtgttagcagctacttagcctggtaccaacagaaacctggccaggctcccaggctcctcatctatgatgcatccaacagggccactggcatcccagccaggttcagtggcagtgggtctgggacagacttcactctcaccatcagcagcctagagcctgaagattttgcagtttattactgtcagcagcgtagcaactggccgatcaccttcggccaagggacacgactggagattaaagagagcaagtacggaccgccctgccccccttgccctgcccccgagttcgagggcggacccagcgtgttcctgttcccccccaagcccaaggacaccctgatgatcagccggacccccgaggtgacctgcgtggtggtggacgtgagccaggaagatcccgaggtccagttcaattggtacgtggacggcgtggaagtgcacaacgccaagaccaagcccagagaggaacagttccaaagcacctaccgggtggtgtctgtgctgaccgtgctgcaccaggactggctgaacggcaaagaatacaagtgcaaggtgtccaacaagggcctgcccagcagcatcgaaaagaccatcagcaaggccaagggccagcctcgcgagccccaggtgtacaccctgcctccctcccaggaagagatgaccaagaaccaggtgtccctgacctgcctggtgaagggcttctaccccagcgacatcgccgtggagtgggagagcaacggccagcctgagaacaactacaagaccacccctcccgtgctggacagcgacggcagcttcttcctgtacagccggctgaccgtggacaagagccggtggcaggaaggcaacgtctttagctgcagcgtgatgcacgaggccctgcacaaccactacacccagaagagcctgagcctgtccctgggcaagttttgggtgctggtggtggttggtggagtcctggcttgctatagcttgctagtaacagtggcctttattattttctgggtgaggagtaagaggagcaggctcctgcacagtgactacatgaacatgactccccgccgccccgggcccacccgcaagcattaccagccctatgccccaccacgcgacttcgcagcctatcgctccaaacggggcagaaagaaactcctgtatatattcaaacaaccatttatgagaccagtacaaactactcaagaggaagatggctgtagctgccgatttccagaagaagaagaaggaggatgtgaactgagagtgaagttcagcaggagcgcagacgcccccgcgtacaagcagggccagaaccagctctataacgagctcaatctaggacgaagagaggagtacgatgttttggacaagagacgtggccgggaccctgagatggggggaaagccgagaaggaagaaccctcaggaaggcctgtacaatgaactgcagaaagataagatggcggaggcctacagtgagattgggatgaaaggcgagcgccggaggggcaaggggcacgatggcctttaccagggtctcagtacagccaccaaggacacctacgacgcccttcacatgcaggccctgccccctcgctaa

SEQ ID NO: 33 - protein, 119 aa, synthetic construct
  REGION 1..119: note = VH
QVQLVQSGAEVKKPGSSVKVSCKASGYAFSYSWINWVRQAPGQGLEWMGRIFPGDGDTDYNGKFKGRVTITADKSTSTAYMELSSLRSEDTAVYYCARNVFDGYWLVYWGQGTLVTVSS

SEQ ID NO: 34 - DNA, 357 bp, synthetic construct
  misc_feature 1..357: note = VH
  source 1..357: mol_type = other DNA
caggtgcaattggtgcagtctggcgctgaagttaagaagcctgggagttcagtgaaggtctcctgcaaggcttccggatacgccttcagctattcttggatcaattgggtgcggcaggcgcctggacaagggctcgagtggatgggacggatctttcccggcgatggggatactgactacaatgggaaattcaagggcagagtcacaattaccgccgacaaatccactagcacagcctatatggagctgagcagcctgagatctgaggacacggccgtgtattactgtgcaagaaatgtctttgatggttactggcttgtttactggggccagggaaccctggtcaccgtctcctca

SEQ ID NO: 35 - protein, 115 aa, synthetic construct
  REGION 1..115: note = VL
DIVMTQTPLSLPVTPGEPASISCRSSKSLLHSNGITYLYWYLQKPGQSPQLLIYQMSNLVSGVPDRFSGSGSGTDFTLKISRVEAEDVGVYYCAQNLELPYTFGGGTKVEIKRTV

SEQ ID NO: 36 - DNA, 345 bp, synthetic construct
  misc_feature 1..345: note = VL
  source 1..345: mol_type = other DNA
gatatcgtgatgacccagactccactctccctgcccgtcacccctggagagcccgccagcattagctgcaggtctagcaagagcctcttgcacagcaatggcatcacttatttgtattggtacctgcaaaagccagggcagtctccacagctcctgatttatcaaatgtccaaccttgtctctggcgtccctgaccggttctccggctccgggtcaggcactgatttcacactgaaaatcagcagggtggaggctgaggatgttggagtttattactgcgctcagaatctagaacttccttacaccttcggcggagggaccaaggtggagatcaaacgtacggtg

SEQ ID NO: 37 - protein, 27 aa, synthetic construct
  REGION 1..27: note = TM
FWVLVVVGGVLACYSLLVTVAFIIFWV

SEQ ID NO: 38 - DNA, 81 bp, synthetic construct
  misc_feature 1..81: note = TM
  source 1..81: mol_type = other DNA
ttttgggtgctggtggtggttggtggagtcctggcttgctatagcttgctagtaacagtggcctttattattttctgggtg

SEQ ID NO: 39 - protein, 41 aa, synthetic construct
  REGION 1..41: note = CS
RSKRSRLLHSDYMNMTPRRPGPTRKHYQPYAPPRDFAAYRS

SEQ ID NO: 40 - DNA, 123 bp, synthetic construct
  misc_feature 1..123: note = CS
  source 1..123: mol_type = other DNA
aggagtaagaggagcaggctcctgcacagtgactacatgaacatgactccccgccgccccgggcccacccgcaagcattaccagccctatgccccaccacgcgacttcgcagcctatcgctcc